European Patent Application EP 4 659 752 A1, published December 10, 2025. Title: Antisense oligonucleotides (ASO) pharmaceutical composition for preventing or treating Avellino corneal dystrophy. Applicant: MediciBIO Co., Ltd. Application WO. The sequence listing filed with the application follows.

SEQUENCE LISTING (67 sequences)

SEQ ID NO: 1 - DNA, 18 bp, synthetic construct
  source 1..18: mol_type = other DNA
ccgtgtggtccgtgtaca

SEQ ID NO: 2 - DNA, 18 bp, synthetic construct
  source 1..18: mol_type = other DNA
tccgtgtggtccgtgtac

SEQ ID NO: 3 - DNA, 18 bp, synthetic construct
  source 1..18: mol_type = other DNA
ctccgtgtggtccgtgta

SEQ ID NO: 4 - DNA, 18 bp, synthetic construct
  source 1..18: mol_type = other DNA
tctccgtgtggtccgtgt

SEQ ID NO: 5 - DNA, 18 bp, synthetic construct
  source 1..18: mol_type = other DNA
ttctccgtgtggtccgtg

SEQ ID NO: 6 - DNA, 18 bp, synthetic construct
  source 1..18: mol_type = other DNA
cttctccgtgtggtccgt

SEQ ID NO: 7 - DNA, 18 bp, synthetic construct
  source 1..18: mol_type = other DNA
gcttctccgtgtggtccg

SEQ ID NO: 8 - DNA, 18 bp, synthetic construct
  source 1..18: mol_type = other DNA
agcttctccgtgtggtcc

SEQ ID NO: 9 - DNA, 18 bp, synthetic construct
  source 1..18: mol_type = other DNA
cagcttctccgtgtggtc

SEQ ID NO: 10 - DNA, 18 bp, synthetic construct
  source 1..18: mol_type = other DNA
ccgtgtggtccgtgtaca

SEQ ID NO: 11 - DNA, 18 bp, synthetic construct
  source 1..18: mol_type = other DNA
tccgtgtggtccgtgtac

SEQ ID NO: 12 - DNA, 18 bp, synthetic construct
  source 1..18: mol_type = other DNA
ctccgtgtggtccgtgta

SEQ ID NO: 13 - DNA, 18 bp, synthetic construct
  source 1..18: mol_type = other DNA
tctccgtgtggtccgtgt

SEQ ID NO: 14 - DNA, 18 bp, synthetic construct
  source 1..18: mol_type = other DNA
ttctccgtgtggtccgtg

SEQ ID NO: 15 - DNA, 18 bp, synthetic construct
  source 1..18: mol_type = other DNA
cttctccgtgtggtccgt

SEQ ID NO: 16 - DNA, 18 bp, synthetic construct
  source 1..18: mol_type = other DNA
gcttctccgtgtggtccg

SEQ ID NO: 17 - DNA, 18 bp, synthetic construct
  source 1..18: mol_type = other DNA
agcttctccgtgtggtcc

SEQ ID NO: 18 - DNA, 18 bp, synthetic construct
  source 1..18: mol_type = other DNA
cagcttctccgtgtggtc

SEQ ID NO: 19 - DNA, 19 bp, synthetic construct
  source 1..19: mol_type = other DNA
ccgtgtggtccgtgtacag

SEQ ID NO: 20 - DNA, 19 bp, synthetic construct
  source 1..19: mol_type = other DNA
tccgtgtggtccgtgtaca

SEQ ID NO: 21 - DNA, 19 bp, synthetic construct
  source 1..19: mol_type = other DNA
ctccgtgtggtccgtgtac

SEQ ID NO: 22 - DNA, 19 bp, synthetic construct
  source 1..19: mol_type = other DNA
tctccgtgtggtccgtgta

SEQ ID NO: 23 - DNA, 19 bp, synthetic construct
  source 1..19: mol_type = other DNA
ttctccgtgtggtccgtgt

SEQ ID NO: 24 - DNA, 19 bp, synthetic construct
  source 1..19: mol_type = other DNA
cttctccgtgtggtccgtg

SEQ ID NO: 25 - DNA, 19 bp, synthetic construct
  source 1..19: mol_type = other DNA
gcttctccgtgtggtccgt

SEQ ID NO: 26 - DNA, 19 bp, synthetic construct
  source 1..19: mol_type = other DNA
agcttctccgtgtggtccg

SEQ ID NO: 27 - DNA, 19 bp, synthetic construct
  source 1..19: mol_type = other DNA
cagcttctccgtgtggtcc

SEQ ID NO: 28 - DNA, 19 bp, synthetic construct
  source 1..19: mol_type = other DNA
tcagcttctccgtgtggtc

SEQ ID NO: 29 - DNA, 19 bp, synthetic construct
  source 1..19: mol_type = other DNA
ccgtgtggtccgtgtacag

SEQ ID NO: 30 - DNA, 19 bp, synthetic construct
  source 1..19: mol_type = other DNA
tccgtgtggtccgtgtaca

SEQ ID NO: 31 - DNA, 19 bp, synthetic construct
  source 1..19: mol_type = other DNA
ctccgtgtggtccgtgtac

SEQ ID NO: 32 - DNA, 19 bp, synthetic construct
  source 1..19: mol_type = other DNA
tctccgtgtggtccgtgta

SEQ ID NO: 33 - DNA, 19 bp, synthetic construct
  source 1..19: mol_type = other DNA
ttctccgtgtggtccgtgt

SEQ ID NO: 34 - DNA, 19 bp, synthetic construct
  source 1..19: mol_type = other DNA
cttctccgtgtggtccgtg

SEQ ID NO: 35 - DNA, 19 bp, synthetic construct
  source 1..19: mol_type = other DNA
gcttctccgtgtggtccgt

SEQ ID NO: 36 - DNA, 19 bp, synthetic construct
  source 1..19: mol_type = other DNA
agcttctccgtgtggtccg

SEQ ID NO: 37 - DNA, 19 bp, synthetic construct
  source 1..19: mol_type = other DNA
cagcttctccgtgtggtcc

SEQ ID NO: 38 - DNA, 19 bp, synthetic construct
  source 1..19: mol_type = other DNA
tcagcttctccgtgtggtc

SEQ ID NO: 39 - DNA, 20 bp, synthetic construct
  source 1..20: mol_type = other DNA
ccgtgtggtccgtgtacagc

SEQ ID NO: 40 - DNA, 20 bp, synthetic construct
  source 1..20: mol_type = other DNA
tccgtgtggtccgtgtacag

SEQ ID NO: 41 - DNA, 20 bp, synthetic construct
  source 1..20: mol_type = other DNA
ctccgtgtggtccgtgtaca

SEQ ID NO: 42 - DNA, 20 bp, synthetic construct
  source 1..20: mol_type = other DNA
tctccgtgtggtccgtgtac

SEQ ID NO: 43 - DNA, 20 bp, synthetic construct
  source 1..20: mol_type = other DNA
ttctccgtgtggtccgtgta

SEQ ID NO: 44 - DNA, 20 bp, synthetic construct
  source 1..20: mol_type = other DNA
cttctccgtgtggtccgtgt

SEQ ID NO: 45 - DNA, 20 bp, synthetic construct
  source 1..20: mol_type = other DNA
gcttctccgtgtggtccgtg

SEQ ID NO: 46 - DNA, 20 bp, synthetic construct
  source 1..20: mol_type = other DNA
agcttctccgtgtggtccgt

SEQ ID NO: 47 - DNA, 20 bp, synthetic construct
  source 1..20: mol_type = other DNA
cagcttctccgtgtggtccg

SEQ ID NO: 48 - DNA, 20 bp, synthetic construct
  source 1..20: mol_type = other DNA
tcagcttctccgtgtggtcc

SEQ ID NO: 49 - DNA, 20 bp, synthetic construct
  source 1..20: mol_type = other DNA
ctcagcttctccgtgtggtc

SEQ ID NO: 50 - DNA, 20 bp, synthetic construct
  source 1..20: mol_type = other DNA
ccgtgtggtccgtgtacagc

SEQ ID NO: 51 - DNA, 20 bp, synthetic construct
  source 1..20: mol_type = other DNA
tccgtgtggtccgtgtacag

SEQ ID NO: 52 - DNA, 20 bp, synthetic construct
  source 1..20: mol_type = other DNA
ctccgtgtggtccgtgtaca

SEQ ID NO: 53 - DNA, 20 bp, synthetic construct
  source 1..20: mol_type = other DNA
tctccgtgtggtccgtgtac

SEQ ID NO: 54 - DNA, 20 bp, synthetic construct
  source 1..20: mol_type = other DNA
ttctccgtgtggtccgtgta

SEQ ID NO: 55 - DNA, 20 bp, synthetic construct
  source 1..20: mol_type = other DNA
cttctccgtgtggtccgtgt

SEQ ID NO: 56 - DNA, 20 bp, synthetic construct
  source 1..20: mol_type = other DNA
gcttctccgtgtggtccgtg

SEQ ID NO: 57 - DNA, 20 bp, synthetic construct
  source 1..20: mol_type = other DNA
agcttctccgtgtggtccgt

SEQ ID NO: 58 - DNA, 20 bp, synthetic construct
  source 1..20: mol_type = other DNA
cagcttctccgtgtggtccg

SEQ ID NO: 59 - DNA, 20 bp, synthetic construct
  source 1..20: mol_type = other DNA
tcagcttctccgtgtggtcc

SEQ ID NO: 60 - DNA, 20 bp, synthetic construct
  source 1..20: mol_type = other DNA
ctcagcttctccgtgtggtc

SEQ ID NO: 61 - DNA, 18 bp, synthetic construct
  source 1..18: mol_type = other DNA
ttctcggtgtggtccgtg

SEQ ID NO: 62 - DNA, 18 bp, synthetic construct
  source 1..18: mol_type = other DNA
ttctccctgtggtccgtg

SEQ ID NO: 63 - DNA, 18 bp, synthetic construct
  source 1..18: mol_type = other DNA
ttctccgagtggtccgtg

SEQ ID NO: 64 - DNA, 18 bp, synthetic construct
  source 1..18: mol_type = other DNA
ttctccgtctggtccgtg

SEQ ID NO: 65 - DNA, 18 bp, synthetic construct
  source 1..18: mol_type = other DNA
ttctccgtgtcgtccgtg

SEQ ID NO: 66 - DNA, 18 bp, synthetic construct
  source 1..18: mol_type = other DNA
ttctccgtgtgctccgtg

SEQ ID NO: 67 - DNA, 18 bp, synthetic construct
  source 1..18: mol_type = other DNA
ttctccgtgtggaccgtg